European Patent Application EP 4 674 964 A1, published January 7, 2026. Title: RNA interference strategies targeting small heat shock protein B8. Applicant: Universiteit Antwerpen. Application EP. The sequence listing filed with the application follows.

SEQUENCE LISTING (24 sequences)

SEQ ID NO: 1 - RNA, 888 nt, synthetic construct
  source 1..888: mol_type = other RNA
gatgccagtactggcccatccttgttttgtccccaaccctagggcttctctgattccaggatacattactttagctgaactcagatttagtgcaagtaaaatgttagagggtgcgggggtgaggactgaccacagattccctggatagtgtagtggtagatttctccacaggatagcgcaattggcaaatcatgcttggttgtgttaggccaaaatactagttttgctttctttaccttttctatcttgatgaaaatgttgcacattctatagttgcaaaacacataaaaggggacttaacatttcacgttgtatcttacttgcagtgaatgcaagggttacttttctctggggacctcccccatcacccaggttcctactctgggctcccgattcccatggctcccaaaccatgccgcatggtttggttaatgaaacccagtagctaaccccactgtgcttccacatgcctggcctaaaatgggtgatatacaggtcttatatccccatatggaatttatccatcaaccacataaaaacaaacagtgccttctgccctctgcccagatgtgtccagcacgttctcaaagtttccacattagcactccctaaggacgctgggagcctgtcagtttatgatctgacctaggtcccccctttcttctgtcccctgtgtttaagtcgggatttttacagagggagctgtctccagacagctccatcaggaaccaagcaaaggccagatagcctgacagataggctagtggtattgtgtatatgggcgggacgtgtgtgtcattattatttgagttatgctgttgtttaggggtaaataacagtaaataattaataataataataataataataaaggagctgacgttctta

SEQ ID NO: 2 - RNA, 20 nt, synthetic construct
  source 1..20: mol_type = other RNA
aggaaccaagcaaaggccag

SEQ ID NO: 3 - RNA, 21 nt, synthetic construct
  source 1..21: mol_type = other RNA
aaggaaccaagcaaaggccag

SEQ ID NO: 4 - DNA, 48 bp, synthetic construct
  source 1..48: mol_type = other DNA
aaggaaccaagcaaaggccagctcgagctggcctttgcttggttcctt

SEQ ID NO: 5 - RNA, 50 nt, synthetic construct
  source 1..50: mol_type = other RNA
  misc_difference 49..50: replace
aaggaaccaagcaaaggccagctcgagctggcctttgcttggttcctttt

SEQ ID NO: 6 - DNA, 21 bp, synthetic construct
  source 1..21: mol_type = other DNA
  misc_difference 1..2: replace
aatctgtctctctgagcctct

SEQ ID NO: 7 - DNA, 21 bp, synthetic construct
  source 1..21: mol_type = other DNA
  misc_difference 1..2: replace
aagatggctttggcatggacc

SEQ ID NO: 8 - DNA, 21 bp, synthetic construct
  source 1..21: mol_type = other DNA
  misc_difference 1: replace
aaggaaccaagcaaaggccag

SEQ ID NO: 9 - DNA, 21 bp, synthetic construct
  source 1..21: mol_type = other DNA
gcttggttgatgggactcatt

SEQ ID NO: 10 - DNA, 21 bp, synthetic construct
  source 1..21: mol_type = other DNA
ccactgtatttgcctcgcttt

SEQ ID NO: 11 - DNA, 21 bp, synthetic construct
  source 1..21: mol_type = other DNA
gccttggaaagtgtgtgtcaa

SEQ ID NO: 12 - DNA, 21 bp, synthetic construct
  source 1..21: mol_type = other DNA
gtggaagtttcaggcaaacat

SEQ ID NO: 13 - DNA, 21 bp, synthetic construct
  source 1..21: mol_type = other DNA
atctctatcgcctcgtcttgt

SEQ ID NO: 14 - DNA, 21 bp, synthetic construct
  source 1..21: mol_type = other DNA
ccaccgtacttgcctagcatt

SEQ ID NO: 15 - DNA, 23 bp, synthetic construct
  source 1..23: mol_type = other DNA
cagaggagttgatggtgaagacc

SEQ ID NO: 16 - DNA, 22 bp, synthetic construct
  source 1..22: mol_type = other DNA
actgtcacaggatccacctctg

SEQ ID NO: 17 - DNA, 21 bp, synthetic construct
  source 1..21: mol_type = other DNA
tgacactggcaaaacaatgca

SEQ ID NO: 18 - DNA, 21 bp, synthetic construct
  source 1..21: mol_type = other DNA
ggtccttttcaccagcaagct

SEQ ID NO: 19 - DNA, 20 bp, synthetic construct
  source 1..20: mol_type = other DNA
tgcaccaccaactgcttagc

SEQ ID NO: 20 - DNA, 21 bp, synthetic construct
  source 1..21: mol_type = other DNA
ggcatggactgtggtcatgag

SEQ ID NO: 21 - RNA, 849 nt, synthetic construct
  source 1..849: mol_type = other RNA
gacgtcagccttggtccttcttcgctcccatccccagccccagggactctctgatttgagggtacactactttagcagcactcagatttaaggcaactcagatgttgggggatgggagggagaaccgaacgaccgtccctggatgatgtagtaatagatttctccacagggtgacgcaatgggtcagccttgcttggttgcgttaggtcaaaggattgggaggtttttcttcatcttatctgggtgaagacgtctcgcagtctacagttgcaaaacaagcaaatggggactgaagatttcatgttaaatttttaccttgcagttaatgcaagagttgcttttctctggggaccttcccatcacccagatccctgctctggaccctccttctacgtggcttggttgatgggactcattggctcacctcagtgtgtttctaaactctttgtctagaagaggttatgggcaggtcttatatccccatatgggatttatccttcaccacacaacacagtgccttttttttgcagcatgaccccatggctctcaaaccatcaccaccaagaactctgggagcccctcagttaattctctggctaaggtccccctttattgtgtcccctgtgtccaagtcacatttttacagagagctgtcttggagcagctccgcaaggaaccaagcaaaggccagacagcctgcacgcaggctagtggcattgtgtgtgtgtttgaggggtggggaggatgtgtgtgtctttgttgtgtgaattgtgctgttgtttagagggaaaataacggtgaataataatgatgataataaaggagctgatgttcttagcaaaaaaaaaa

SEQ ID NO: 22 - protein, 196 aa, Homo sapiens
MADGQMPFSCHYPSRLRRDPFRDSPLSSRLLDDGFGMDPFPDDLTASWPDWALPRLSSAWPGTLRSGMVPRGPTATARFGVPAEGRTPPPFPGEPWKVCVNVHSFKPEELMVKTKDGYVEVSGKHEEKQQEGGIVSKNFTKKIQLPAEVDPVTVFASLSPEGLLIIEAPQVPPYSTFGESSFNNELPQDSQEVTCT

SEQ ID NO: 23 - DNA, 448 bp, synthetic construct
  source 1..448: mol_type = other DNA
ctgcgctctcaggcacgacacgactcctccgctgcccaccgcagactgaggcagcgctgagtcgccggcgccgcagcgcagatggtcgcgcccgtgcccccctatctcgcgcctcgcgtggtgcggtccggctgggccggcggcggcgcggacgcgaccaaggtggccgggaaggggagtttgcgggggaccggcgagtgacgtcagcgcgccttcagtgctgaggcggcggtggcgcgcgccgccaggcgggggcgaaggcactgtccgcggtgctgaagctggcagtgcgcacgcgcctcgccgcatcctgtttcccctccccctctctgataggggatgcgcaatttggggaatgggggttgggtgcttgtccagtgggtcggggtcggtcgtcaggtaggcacccccaccccgcctcatcctggtcctaaaacccacttgcact

SEQ ID NO: 24 - DNA, 380 bp, synthetic construct
  source 1..380: mol_type = other DNA
ggcattgattattgactagttattaatagtaatcaattacggggtcattagttcatagcccatatatggagttccgcgttacataacttacggtaaatggcccgcctggctgaccgcccaacgacccccgcccattgacgtcaataatgacgtatgttcccatagtaacgccaatagggactttccattgacgtcaatgggtggagtatttacggtaaactgcccacttggcagtacatcaagtgtatcatatgccaagtccgccccctattgacgtcaatgacggtaaatggcccgcctggcattatgcccagtacatgaccttacgggactttcctacttggcagtacatctacgtattagtcatcgctattaccatg